European Patent Application EP 4 588 489 A1, published July 23, 2025. Title: LINKER FOR ANTIBODY-DRUG CONJUGATE AND USE THEREOF. Applicant: SHANGHAI JUNSHI BIOSCIENCES CO., LTD. Application CN. The sequence listing filed with the application follows.

SEQUENCE LISTING (6 sequences)

SEQ ID NO: 1 - protein, 214 aa, synthetic construct
DIQLTQSPSSLSASVGDRVSITCKASQDVSIAVAWYQQKPGKAPKLLIYSASYRYTGVPDRFSGSGSGTDFTLTISSLQPEDFAVYYCQQHYITPLTFGAGTKVEIKRTVAAPSVFIFPPSDEQLKSGTASVVCLLNNFYPREAKVQWKVDNALQSGNSQESVTEQDSKDSTYSLSSTLTLSKADYEKHKVYACEVTHQGLSSPVTKSFNRGEC

SEQ ID NO: 2 - protein, 451 aa, synthetic construct
QVQLQQSGSELKKPGASVKVSCKASGYTFTNYGMNWVKQAPGQGLKWMGWINTYTGEPTYTDDFKGRFAFSLDTSVSTAYLQISSLKADDTAVYFCARGGFGSSYWYFDVWGQGSLVTVSSASTKGPSVFPLAPSSKSTSGGTAALGCLVKDYFPEPVTVSWNSGALTSGVHTFPAVLQSSGLYSLSSVVTVPSSSLGTQTYICNVNHKPSNTKVDKRVEPKSCDKTHTCPPCPAPELLGGPSVFLFPPKPKDTLMISRTPEVTCVVVDVSHEDPEVKFNWYVDGVEVHNAKTKPREEQYNSTYRVVSVLTVLHQDWLNGKEYKCKVSNKALPAPIEKTISKAKGQPREPQVYTLPPSREEMTKNQVSLTCLVKGFYPSDIAVEWESNGQPENNYKTTPPVLDSDGSFFLYSKLTVDKSRWQQGNVFSCSVMHEALHNHYTQKSLSLSPGK

SEQ ID NO: 3 - protein, 214 aa, synthetic construct
DIQMTQSPSSLSASVGDRVTITCKASQDVSTAVAWYQQKPGKAPKLLIYSASYRYTGVPSRFSGSGSGTDFTLTISSLQPEDFAVYYCQQHYITPLTFGQGTKLEIKRTVAAPSVFIFPPSDEQLKSGTASVVCLLNNFYPREAKVQWKVDNALQSGNSQESVTEQDSKDSTYSLSSTLTLSKADYEKHKVYACEVTHQGLSSPVTKSFNRGEC

SEQ ID NO: 4 - protein, 451 aa, synthetic construct
QVQLVQSGAEVKKPGASVKVSCKASGYTFTTAGMQWVRQAPGQGLEWMGWINTHSGVPKYAEDFKGRVTISADTSTSTAYLQLSSLKSEDTAVYYCARSGFGSSYWYFDVWGQGTLVTVSSASTKGPSVFPLAPSSKSTSGGTAALGCLVKDYFPEPVTVSWNSGALTSGVHTFPAVLQSSGLYSLSSVVTVPSSSLGTQTYICNVNHKPSNTKVDKRVEPKSCDKTHTCPPCPAPELLGGPSVFLFPPKPKDTLMISRTPEVTCVVVDVSHEDPEVKFNWYVDGVEVHNAKTKPREEQYNSTYRVVSVLTVLHQDWLNGKEYKCKVSNKALPAPIEKTISKAKGQPREPQVYTLPPSREEMTKNQVSLTCLVKGFYPSDIAVEWESNGQPENNYKTTPPVLDSDGSFFLYSKLTVDKSRWQQGNVFSCSVMHEALHNHYTQKSLSLSPGK

SEQ ID NO: 5 - protein, 451 aa, synthetic construct
EVQLVESGGGLVKPGGSLRLSCAASGFTFSNFDMAWVRQAPGKGLEWVASIVTRGDDTYYRDSVRGRFTISRDNAKNTQYLQMNSLRAEDTAVYYCARHDYGGPSGWFGYWGQGTLVTVSSASTKGPSVFPLAPSSKSTSGGTAALGCLVKDYFPEPVTVSWNSGALTSGVHTFPAVLQSSGLYSLSSVVTVPSSSLGTQTYICNVNHKPSNTKVDKKVEPKSCDKTHTCPPCPAPELLGGPSVFLFPPKPKDTLMISRTPEVTCVVVDVSHEDPEVKFNWYVDGVEVHNAKTKPREEQYNSTYRVVSVLTVLHQDWLNGKEYKCKVSNKALPAPIEKTISKAKGQPREPQVYTLPPSRDELTKNQVSLTCLVKGFYPSDIAVEWESNGQPENNYKTTPPVLDSDGSFFLYSKLTVDKSRWQQGNVFSCSVMHEALHNHYTQKSLSLSPGK

SEQ ID NO: 6 - protein, 214 aa, synthetic construct
DIQMTQSPSSLSASVGDRVTITCRASQGFSNNLNWYQQKPGKTPKPLIYYTSNLHSGVPSRFSGSGSGTDYSLTISSLQPEDFATYYCQQDASFPPTFGQGTKLEIKRTVAAPSVFIFPPSDEQLKSGTASVVCLLNNFYPREAKVQWKVDNALQSGNSQESVTEQDSKDSTYSLSSTLTLSKADYEKHKVYACEVTHQGLSSPVTKSFNRGEC